European Patent Application EP 4 122 949 A1, published January 25, 2023. Title: MUTANT PORE. Applicant: OXFORD NANOPORE TECHNOLOGIES LIMITED. The sequence listing filed with the application follows.

SEQUENCE LISTING (24 sequences)

SEQ ID NO: 1 - DNA, 897 bp, Eisenia fetida
atgagtgcgaaggctgctgaaggttatgaacaaatcgaagttgatgtggttgctgtgtggaaggaaggttatgtgtatgaaaatcgtggtagtacctccgtggatcaaaaaattaccatcacgaaaggcatgaagaacgttaatagcgaaacccgtacggtcaccgcgacgcattctattggcagtaccatctccacgggtgacgcctttgaaatcggctccgtggaagtttcatattcgcatagccacgaagaatcacaagtttcgatgaccgaaacggaagtctacgaatcaaaagtgattgaacacaccattacgatcccgccgacctcgaagttcacgcgctggcagctgaacgcagatgtcggcggtgctgacattgaatatatgtacctgatcgatgaagttaccccgattggcggtacgcagagtattccgcaagtgatcacctcccgtgcaaaaattatcgttggtcgccagattatcctgggcaagaccgaaattcgtatcaaacatgctgaacgcaaggaatatatgaccgtggttagccgtaaatcttggccggcggccacgctgggtcacagtaaactgtttaagttcgtgctgtacgaagattggggcggttttcgcatcaaaaccctgaatacgatgtattctggttatgaatacgcgtatagctctgaccagggcggtatctacttcgatcaaggcaccgacaacccgaaacagcgttgggccattaataagagcctgccgctgcgccatggtgatgtcgtgacctttatgaacaaatacttcacgcgttctggtctgtgctatgatgacggcccggcgaccaatgtgtattgtctggataaacgcgaagacaagtggattctggaagttgtcggctaatga

SEQ ID NO: 2 - protein, 297 aa, Eisenia fetida
MSAKAAEGYEQIEVDVVAVWKEGYVYENRGSTSVDQKITITKGMKNVNSETRTVTATHSIGSTISTGDAFEIGSVEVSYSHSHEESQVSMTETEVYESKVIEHTITIPPTSKFTRWQLNADVGGADIEYMYLIDEVTPIGGTQSIPQVITSRAKIIVGRQIILGKTEIRIKHAERKEYMTVVSRKSWPAATLGHSKLFKFVLYEDWGGFRIKTLNTMYSGYEYAYSSDQGGIYFDQGTDNPKQRWAINKSLPLRHGDVVTFMNKYFTRSGLCYDDGPATNVYCLDKREDKWILEVVG

SEQ ID NO: 3 - DNA, 1830 bp, Bacteriophage phi-29
atgaaacacatgccgcgtaaaatgtatagctgcgcgtttgaaaccacgaccaaagtggaagattgtcgcgtttgggcctatggctacatgaacatcgaagatcattctgaatacaaaatcggtaacagtctggatgaatttatggcatgggtgctgaaagttcaggcggatctgtacttccacaacctgaaatttgatggcgcattcattatcaactggctggaacgtaatggctttaaatggagcgcggatggtctgccgaacacgtataataccattatctctcgtatgggccagtggtatatgattgatatctgcctgggctacaaaggtaaacgcaaaattcataccgtgatctatgatagcctgaaaaaactgccgtttccggtgaagaaaattgcgaaagatttcaaactgacggttctgaaaggcgatattgattatcacaaagaacgtccggttggttacaaaatcaccccggaagaatacgcatacatcaaaaacgatatccagatcatcgcagaagcgctgctgattcagtttaaacagggcctggatcgcatgaccgcgggcagtgatagcctgaaaggtttcaaagatatcatcacgaccaaaaaattcaaaaaagtgttcccgacgctgagcctgggtctggataaagaagttcgttatgcctaccgcggcggttttacctggctgaacgatcgtttcaaagaaaaagaaattggcgagggtatggtgtttgatgttaatagtctgtatccggcacagatgtacagccgcctgctgccgtatggcgaaccgatcgtgttcgagggtaaatatgtttgggatgaagattacccgctgcatattcagcacatccgttgtgaatttgaactgaaagaaggctatattccgaccattcagatcaaacgtagtcgcttctataagggtaacgaatacctgaaaagctctggcggtgaaatcgcggatctgtggctgagtaacgtggatctggaactgatgaaagaacactacgatctgtacaacgttgaatacatcagcggcctgaaatttaaagccacgaccggtctgttcaaagatttcatcgataaatggacctacatcaaaacgacctctgaaggcgcgattaaacagctggccaaactgatgctgaacagcctgtatggcaaattcgcctctaatccggatgtgaccggtaaagttccgtacctgaaagaaaatggcgcactgggttttcgcctgggcgaagaagaaacgaaagatccggtgtataccccgatgggtgttttcattacggcctgggcacgttacacgaccatcaccgcggcccaggcatgctatgatcgcattatctactgtgataccgattctattcatctgacgggcaccgaaatcccggatgtgattaaagatatcgttgatccgaaaaaactgggttattgggcccacgaaagtacgtttaaacgtgcaaaatacctgcgccagaaaacctacatccaggatatctacatgaaagaagtggatggcaaactggttgaaggttctccggatgattacaccgatatcaaattcagtgtgaaatgcgccggcatgacggataaaatcaaaaaagaagtgaccttcgaaaacttcaaagttggtttcagccgcaaaatgaaaccgaaaccggtgcaggttccgggcggtgtggttctggtggatgatacgtttaccattaaatctggcggtagtgcgtggagccatccgcagttcgaaaaaggcggtggctctggtggcggttctggcggtagtgcctggagccacccgcagtttgaaaaataataa

SEQ ID NO: 4 - protein, 608 aa, Bacteriophage phi-29
MKHMPRKMYSCAFETTTKVEDCRVWAYGYMNIEDHSEYKIGNSLDEFMAWVLKVQADLYFHNLKFDGAFIINWLERNGFKWSADGLPNTYNTIISRMGQWYMIDICLGYKGKRKIHTVIYDSLKKLPFPVKKIAKDFKLTVLKGDIDYHKERPVGYKITPEEYAYIKNDIQIIAEALLIQFKQGLDRMTAGSDSLKGFKDIITTKKFKKVFPTLSLGLDKEVRYAYRGGFTWLNDRFKEKEIGEGMVFDVNSLYPAQMYSRLLPYGEPIVFEGKYVWDEDYPLHIQHIRCEFELKEGYIPTIQIKRSRFYKGNEYLKSSGGEIADLWLSNVDLELMKEHYDLYNVEYISGLKFKATTGLFKDFIDKWTYIKTTSEGAIKQLAKLMLNSLYGKFASNPDVTGKVPYLKENGALGFRLGEEETKDPVYTPMGVFITAWARYTTITAAQACYDRIIYCDTDSIHLTGTEIPDVIKDIVDPKKLGYWAHESTFKRAKYLRQKTYIQDIYMKEVDGKLVEGSPDDYTDIKFSVKCAGMTDKIKKEVTFENFKVGFSRKMKPKPVQVPGGVVLVDDTFTIKSGGSAWSHPQFEKGGGSGGGSGGSAWSHPQFEK

SEQ ID NO: 5 - DNA, 1390 bp, Escherichia coli
atgatgaacgatggcaaacagcagagcaccttcctgtttcatgattatgaaaccttcggtacccatccggccctggatcgtccggcgcagtttgcggccattcgcaccgatagcgaattcaatgtgattggcgaaccggaagtgttttattgcaaaccggccgatgattatctgccgcagccgggtgcggtgctgattaccggtattaccccgcaggaagcgcgcgcgaaaggtgaaaacgaagcggcgtttgccgcgcgcattcatagcctgtttaccgtgccgaaaacctgcattctgggctataacaatgtgcgcttcgatgatgaagttacccgtaatatcttttatcgtaacttttatgatccgtatgcgtggagctggcagcatgataacagccgttgggatctgctggatgtgatgcgcgcgtgctatgcgctgcgcccggaaggcattaattggccggaaaacgatgatggcctgccgagctttcgtctggaacatctgaccaaagccaacggcattgaacatagcaatgcccatgatgcgatggccgatgtttatgcgaccattgcgatggcgaaactggttaaaacccgtcagccgcgcctgtttgattatctgtttacccaccgtaacaaacacaaactgatggcgctgattgatgttccgcagatgaaaccgctggtgcatgtgagcggcatgtttggcgcctggcgcggcaacaccagctgggtggccccgctggcctggcacccggaaaatcgtaacgccgtgattatggttgatctggccggtgatattagcccgctgctggaactggatagcgataccctgcgtgaacgcctgtataccgccaaaaccgatctgggcgataatgccgccgtgccggtgaaactggttcacattaacaaatgcccggtgctggcccaggcgaacaccctgcgcccggaagatgcggatcgtctgggtattaatcgccagcattgtctggataatctgaaaatcctgcgtgaaaacccgcaggtgcgtgaaaaagtggtggcgatcttcgcggaagcggaaccgttcaccccgagcgataacgtggatgcgcagctgtataacggcttctttagcgatgccgatcgcgcggcgatgaaaatcgttctggaaaccgaaccgcgcaatctgccggcgctggatattacctttgttgataaacgtattgaaaaactgctgtttaattatcgtgcgcgcaattttccgggtaccctggattatgccgaacagcagcgttggctggaacatcgtcgtcaggttttcaccccggaatttctgcagggttatgcggatgaactgcagatgctggttcagcagtatgccgatgataaagaaaaagtggcgctgc

SEQ ID NO: 6 - protein, 485 aa, Escherichia coli
MMNDGKQQSTFLFHDYETFGTHPALDRPAQFAAIRTDSEFNVIGEPEVFYCKPADDYLPQPGAVLITGITPQEARAKGENEAAFAARIHSLFTVPKTCILGYNNVRFDDEVTRNIFYRNFYDPYAWSWQHDNSRWDLLDVMRACYALRPEGINWPENDDGLPSFRLEHLTKANGIEHSNAHDAMADVYATIAMAKLVKTRQPRLFDYLFTHRNKHKLMALIDVPQMKPLVHVSGMFGAWRGNTSWVAPLAWHPENRNAVIMVDLAGDISPLLELDSDTLRERLYTAKTDLGDNAAVPVKLVHINKCPVLAQANTLRPEDADRLGINRQHCLDNLKILRENPQVREKVVAIFAEAEPFTPSDNVDAQLYNGFFSDADRAAMKIVLETEPRNLPALDITFVDKRIEKLLFNYRARNFPGTLDYAEQQRWLEHRRQVFTPEFLQGYADELQMLVQQYADDKEKVALLKALWQYAEEIVSGSGHHHHHH

SEQ ID NO: 7 - DNA, 804 bp, Escherichia coli
atgaaatttgtctcttttaatatcaacggcctgcgcgccagacctcaccagcttgaagccatcgtcgaaaagcaccaaccggatgtgattggcctgcaggagacaaaagttcatgacgatatgtttccgctcgaagaggtggcgaagctcggctacaacgtgttttatcacgggcagaaaggccattatggcgtggcgctgctgaccaaagagacgccgattgccgtgcgtcgcggctttcccggtgacgacgaagaggcgcagcggcggattattatggcggaaatcccctcactgctgggtaatgtcaccgtgatcaacggttacttcccgcagggtgaaagccgcgaccatccgataaaattcccggcaaaagcgcagttttatcagaatctgcaaaactacctggaaaccgaactcaaacgtgataatccggtactgattatgggcgatatgaatatcagccctacagatctggatatcggcattggcgaagaaaaccgtaagcgctggctgcgtaccggtaaatgctctttcctgccggaagagcgcgaatggatggacaggctgatgagctgggggttggtcgataccttccgccatgcgaatccgcaaacagcagatcgtttctcatggtttgattaccgctcaaaaggttttgacgataaccgtggtctgcgcatcgacctgctgctcgccagccaaccgctggcagaatgttgcgtagaaaccggcatcgactatgaaatccgcagcatggaaaaaccgtccgatcacgcccccgtctgggcgaccttccgccgc

SEQ ID NO: 8 - protein, 268 aa, Escherichia coli
MKFVSFNINGLRARPHQLEAIVEKHQPDVIGLQETKVHDDMFPLEEVAKLGYNVFYHGQKGHYGVALLTKETPIAVRRGFPGDDEEAQRRIIMAEIPSLLGNVTVINGYFPQGESRDHPIKFPAKAQFYQNLQNYLETELKRDNPVLIMGDMNISPTDLDIGIGEENRKRWLRTGKCSFLPEEREWMDRLMSWGLVDTFRHANPQTADRFSWFDYRSKGFDDNRGLRIDLLLASQPLAECCVETGIDYEIRSMEKPSDHAPVWATFRR

SEQ ID NO: 9 - DNA, 1275 bp, Thermus thermophilus
atgtttcgtcgtaaagaagatctggatccgccgctggcactgctgccgctgaaaggcctgcgcgaagccgccgcactgctggaagaagcgctgcgtcaaggtaaacgcattcgtgttcacggcgactatgatgcggatggcctgaccggcaccgcgatcctggttcgtggtctggccgccctgggtgcggatgttcatccgtttatcccgcaccgcctggaagaaggctatggtgtcctgatggaacgcgtcccggaacatctggaagcctcggacctgtttctgaccgttgactgcggcattaccaaccatgcggaactgcgcgaactgctggaaaatggcgtggaagtcattgttaccgatcatcatacgccgggcaaaacgccgccgccgggtctggtcgtgcatccggcgctgacgccggatctgaaagaaaaaccgaccggcgcaggcgtggcgtttctgctgctgtgggcactgcatgaacgcctgggcctgccgccgccgctggaatacgcggacctggcagccgttggcaccattgccgacgttgccccgctgtggggttggaatcgtgcactggtgaaagaaggtctggcacgcatcccggcttcatcttgggtgggcctgcgtctgctggctgaagccgtgggctataccggcaaagcggtcgaagtcgctttccgcatcgcgccgcgcatcaatgcggcttcccgcctgggcgaagcggaaaaagccctgcgcctgctgctgacggatgatgcggcagaagctcaggcgctggtcggcgaactgcaccgtctgaacgcccgtcgtcagaccctggaagaagcgatgctgcgcaaactgctgccgcaggccgacccggaagcgaaagccatcgttctgctggacccggaaggccatccgggtgttatgggtattgtggcctctcgcatcctggaagcgaccctgcgcccggtctttctggtggcccagggcaaaggcaccgtgcgttcgctggctccgatttccgccgtcgaagcactgcgcagcgcggaagatctgctgctgcgttatggtggtcataaagaagcggcgggtttcgcaatggatgaagcgctgtttccggcgttcaaagcacgcgttgaagcgtatgccgcacgtttcccggatccggttcgtgaagtggcactgctggatctgctgccggaaccgggcctgctgccgcaggtgttccgtgaactggcactgctggaaccgtatggtgaaggtaacccggaaccgctgttcctg

SEQ ID NO: 10 - protein, 425 aa, Thermus thermophilus
MFRRKEDLDPPLALLPLKGLREAAALLEEALRQGKRIRVHGDYDADGLTGTAILVRGLAALGADVHPFIPHRLEEGYGVLMERVPEHLEASDLFLTVDCGITNHAELRELLENGVEVIVTDHHTPGKTPPPGLVVHPALTPDLKEKPTGAGVAFLLLWALHERLGLPPPLEYADLAAVGTIADVAPLWGWNRALVKEGLARIPASSWVGLRLLAEAVGYTGKAVEVAFRIAPRINAASRLGEAEKALRLLLTDDAAEAQALVGELHRLNARRQTLEEAMLRKLLPQADPEAKAIVLLDPEGHPGVMGIVASRILEATLRPVFLVAQGKGTVRSLAPISAVEALRSAEDLLLRYGGHKEAAGFAMDEALFPAFKARVEAYAARFPDPVREVALLDLLPEPGLLPQVFRELALLEPYGEGNPEPLFL

SEQ ID NO: 11 - DNA, 738 bp, Bacteriophage lambda
tccggaagcggctctggtagtggttctggcatgacaccggacattatcctgcagcgtaccgggatcgatgtgagagctgtcgaacagggggatgatgcgtggcacaaattacggctcggcgtcatcaccgcttcagaagttcacaacgtgatagcaaaaccccgctccggaaagaagtggcctgacatgaaaatgtcctacttccacaccctgcttgctgaggtttgcaccggtgtggctccggaagttaacgctaaagcactggcctggggaaaacagtacgagaacgacgccagaaccctgtttgaattcacttccggcgtgaatgttactgaatccccgatcatctatcgcgacgaaagtatgcgtaccgcctgctctcccgatggtttatgcagtgacggcaacggccttgaactgaaatgcccgtttacctcccgggatttcatgaagttccggctcggtggtttcgaggccataaagtcagcttacatggcccaggtgcagtacagcatgtgggtgacgcgaaaaaatgcctggtactttgccaactatgacccgcgtatgaagcgtgaaggcctgcattatgtcgtgattgagcgggatgaaaagtacatggcgagttttgacgagatcgtgccggagttcatcgaaaaaatggacgaggcactggctgaaattggttttgtatttggggagcaatggcgatctggctctggttccggcagcggttccgga

SEQ ID NO: 12 - protein, 226 aa, Bacteriophage lambda
MTPDIILQRTGIDVRAVEQGDDAWHKLRLGVITASEVHNVIAKPRSGKKWPDMKMSYFHTLLAEVCTGVAPEVNAKALAWGKQYENDARTLFEFTSGVNVTESPIIYRDESMRTACSPDGLCSDGNGLELKCPFTSRDFMKFRLGGFEAIKSAYMAQVQYSMWVTRKNAWYFANYDPRMKREGLHYVVIERDEKYMASFDEIVPEFIEKMDEALAEIGFVFGEQWR

SEQ ID NO: 13 - protein, 760 aa, Methanococcoides burtonii
MMIRELDIPRDIIGFYEDSGIKELYPPQAEAIEMGLLEKKNLLAAIPTASGKTLLAELAMIKAIREGGKALYIVPLRALASEKFERFKELAPFGIKVGISTGDLDSRADWLGVNDIIVATSEKTDSLLRNGTSWMDEITTVVVDEIHLLDSKNRGPTLEVTITKLMRLNPDVQVVALSATVGNAREMADWLGAALVLSEWRPTDLHEGVLFGDAINFPGSQKKIDRLEKDDAVNLVLDTIKAEGQCLVFESSRRNCAGFAKTASSKVAKILDNDIMIKLAGIAEEVESTGETDTAIVLANCIRKGVAFHHAGLNSNHRKLVENGFRQNLIKVISSTPTLAAGLNLPARRVIIRSYRRFDSNFGMQPIPVLEYKQMAGRAGRPHLDPYGESVLLAKTYDEFAQLMENYVEADAEDIWSKLGTENALRTHVLSTIVNGFASTRQELFDFFGATFFAYQQDKWMLEEVINDCLEFLIDKAMVSETEDIEDASKLFLRGTRLGSLVSMLYIDPLSGSKIVDGFKDIGKSTGGNMGSLEDDKGDDITVTDMTLLHLVCSTPDMRQLYLRNTDYTIVNEYIVAHSDEFHEIPDKLKETDYEWFMGEVKTAMLLEEWVTEVSAEDITRHFNVGEGDIHALADTSEWLMHAAAKLAELLGVEYSSHAYSLEKRIRYGSGLDLMELVGIRGVGRVRARKLYNAGFVSVAKLKGADISVLSKLVGPKVAYNILSGIGVRVNDKHFNSAPISSNTLDTLLDKNQKTFNDFQ

SEQ ID NO: 14 - protein, 300 aa, Eisenia fetida
MSSSTVMADGFEEIEVDVVSVWKEGYAYENRGNSSVQQKITMTKGMKNLNSETKTLTATHTLGRTLKVGDPFEIASVEVSYTFSHQKSQVSMTQTEVYSSQVIEHTVTIPPNKKFTRWKLNADVGGTGIEYMYLIDEVTAIGADLTIPEVNKSRAKILVGRQIHLGETEIRIKHAERKEYMTVISRKSWPAATLGNSNLFKFVLFEDSSGIRIKTLNTMYPGYEWAYSSDQGGIYFDESSDNPKQRWALSKAMPLRHGDVVTFRNNFFTNSGMCYDDGPATNVYCLEKREDKWILEVVNT

SEQ ID NO: 15 - protein, 300 aa, Eisenia fetida
MSSRAGIAEGYEQIEVDVVAVWKEGYVYENRGSTSVEQKIKITKGMRNLNSETKTLTASHSIGSTISTGDLFEIATVDVSYSYSHEESQVSMTETEVYESKEIEHTITIPPTSKFTRWQLNADVGGADIEYMYLIDEVTPIGGTLSIPQVIKSRAKILVGREIYLGETEIRIKHADRKEYMTVVSRKSWPAATLGHSKLYKFVLYEDMYGFRIKTLNTMYSGYEYAYSSDQGGIYFDQGSDNPKQRWAINKSLPLRHGDVVTFMNKYFTRSGLCYYDGPATDVYCLDKREDKWILEVVKP

SEQ ID NO: 16 - protein, 300 aa, Eisenia fetida
MSATAVTADGLEEIEVDVVAVWKEGYVYENRGDTSVEQKITMTKGMKNLNSETKTLTATHTVGRTLKVGDPFEIGSVEVSYSFSHQESQVSMTQTEVYSSQVIEHTVTIPPTSKFTRWKLNADVGGTDIEYMYLIDEVTPISVTQTIPQVIRSRAKILVGRQIHLGTTAVRIKHAERQEYMTVIERKKWPAATLGKSNLFKFVLFEDSSGTRIKTLNTMYPGYEWAYSSDQGGVYFDESSDNPKQRWALSKALPLRHGDVVTFMNKYFTNSGLCYDDGPATNVYCLDKREDKWILEVVNP

SEQ ID NO: 17 - protein, 252 aa, Bacillus thuringiensis
MDVIREYLMFNELSALSSSPESVRSRFSSIYGTNPDGIALNNETYFNAVKPPITAQYGYYCYKNVGTVQYVNRPTDINPNVILAQDTLTNNTNEPFTTTITITGSFTNTSTVTSSTTTGFKFTSKLSIKKVFEIGGEVSFSTTIGTSETTTETITVSKSVTVTVPAQSRRTIQLTAKIAKESADFSAPITVDGYFGANFPKRVGPGGHYFWFNPARDVLNTTSGTLRGTVTNVSSFDFQTIVQPARSLLDEQ

SEQ ID NO: 18 - protein, 439 aa, Enterobacteria phage T4
MTFDDLTEGQKNAFNIVMKAIKEKKHHVTINGPAGTGKTTLTKFIIEALISTGETGIILAAPTHAAKKILSKLSGKEASTIHSILKINPVTYEENVLFEQKEVPDLAKCRVLICDEVSMYDRKLFKILLSTIPPWCTIIGIGDNKQIRPVDPGENTAYISPFFTHKDFYQCELTEVKRSNAPIIDVATDVRNGKWIYDKVVDGHGVRGFTGDTALRDFMVNYFSIVKSLDDLFENRVMAFTNKSVDKLNSIIRKKIFETDKDFIVGEIIVMQEPLFKTYKIDGKPVSEIIFNNGQLVRIIEAEYTSTFVKARGVPGEYLIRHWDLTVETYGDDEYYREKIKIISSDEELYKFNLFLGKTAETYKNWNKGGKAPWSDFWDAKSQFSKVKALPASTFHKAQGMSVDRAFIYTPCIHYADVELAQQLLYVGVTRGRYDVFYV

SEQ ID NO: 19 - DNA, 35 bp, Artificial Sequence
  Adaptor portion B of Fig 5
ggcgtctgcttgggtgtttaacctttttttttttt

SEQ ID NO: 20 - DNA, 28 bp, Artificial Sequence
  Adaptor portion D of Fig 5
ggttgtttctgttggtgctgatattgct

SEQ ID NO: 21 - DNA, 20 bp, Artificial Sequence
  Adaptor portion E of Fig 5
aacacccaagcagacgcctt

SEQ ID NO: 22 - DNA, 45 bp, Artificial Sequence
  Adaptor portion F of Fig 5
gcaatatcagcaccaacagaaacaacctttgaggcgagcggtcaa

SEQ ID NO: 23 - DNA, 10178 bp, Artificial Sequence
  10kb Lambda cDNA
caaagtccatgccatcaaactgctggttttcattgatgatgcgggaccagccatcaacgcccaccaccggaacgatgccattctgcttatcaggaaaggcgtaaatttctttcgtccacggattaaggccgtactggttggcaacgatcagtaatgcgatgaactgcgcatcgctggcatcacctttaaatgccgtctggcgaagagtggtgatcagttcctgtgggtcgacagaatccatgccgacacgttcagccagcttcccagccagcgttgcgagtgcagtactcattcgttttatacctctgaatcaatatcaacctggtggtgagcaatggtttcaaccatgtaccggatgtgttctgccatgcgctcctgaaactcaacatcgtcatcaaacgcacgggtaatggattttttgctggccccgtggcgttgcaaatgatcgatgcatagcgattcaaacaggtgctggggcaggcctttttccatgtcgtctgccagttctgcctctttctcttcacgggcgagctgctggtagtgacgcgcccagctctgagcctcaagacgatcctgaatgtaataagcgttcatggctgaactcctgaaatagctgtgaaaatatcgcccgcgaaatgccgggctgattaggaaaacaggaaagggggttagtgaatgcttttgcttgatctcagtttcagtattaatatccattttttataagcgtcgacggcttcacgaaacatcttttcatcgccaataaaagtggcgatagtgaatttagtctggatagccataagtgtttgatccattctttgggactcctggctgattaagtatgtcgataaggcgtttccatccgtcacgtaatttacgggtgattcgttcaagtaaagattcggaagggcagccagcaacaggccaccctgcaatggcatattgcatggtgtgctccttatttatacataacgaaaaacgcctcgagtgaagcgttattggtatgcggtaaaaccgcactcaggcggccttgatagtcatatcatctgaatcaaatattcctgatgtatcgatatcggtaattcttattccttcgctaccatccattggaggccatccttcctgaccatttccatcattccagtcgaactcacacacaacaccatatgcatttaagtcgcttgaaattgctataagcagagcatgttgcgccagcatgattaatacagcatttaatacagagccgtgtttattgagtcggtattcagagtctgaccagaaattattaatctggtgaagtttttcctctgtcattacgtcatggtcgatttcaatttctattgatgctttccagtcgtaatcaatgatgtattttttgatgtttgacatctgttcatatcctcacagataaaaaatcgccctcacactggagggcaaagaagatttccaataatcagaacaagtcggctcctgtttagttacgagcgacattgctccgtgtattcactcgttggaatgaatacacagtgcagtgtttattctgttatttatgccaaaaataaaggccactatcaggcagctttgttgttctgtttaccaagttctctggcaatcattgccgtcgttcgtattgcccatttatcgacatatttcccatcttccattacaggaaacatttcttcaggcttaaccatgcattccgattgcagcttgcatccattgcatcgcttgaattgtccacaccattgatttttatcaatagtcgtagtcatacggatagtcctggtattgttccatcacatcctgaggatgctcttcgaactcttcaaattcttcttccatatatcaccttaaatagtggattgcggtagtaaagattgtgcctgtcttttaaccacatcaggctcggtggttctcgtgtacccctacagcgagaaatcggataaactattacaacccctacagtttgatgagtatagaaatggatccactcgttattctcggacgagtgttcagtaatgaacctctggagagaaccatgtatatgatcgttatctgggttggacttctgcttttaagcccagataactggcctgaatatgttaatgagagaatcggtattcctcatgtgtggcatgttttcgtctttgctcttgcattttcgctagcaattaatgtgcatcgattatcagctattgccagcgccagatataagcgatttaagctaagaaaacgcattaagatgcaaaacgataaagtgcgatcagtaattcaaaaccttacagaagagcaatctatggttttgtgcgcagcccttaatgaaggcaggaagtatgtggttacatcaaaacaattcccatacattagtgagttgattgagcttggtgtgttgaacaaaactttttcccgatggaatggaaagcatatattattccctattgaggatatttactggactgaattagttgccagctatgatccatataatattgagataaagccaaggccaatatctaagtaactagataagaggaatcgattttcccttaattttctggcgtccactgcatgttatgccgcgttcgccaggcttgctgtaccatgtgcgctgattcttgcgctcaatacgttgcaggttgctttcaatctgtttgtggtattcagccagcactgtaaggtctatcggatttagtgcgctttctactcgtgatttcggtttgcgattcagcgagagaatagggcggttaactggttttgcgcttaccccaaccaacaggggatttgctgctttccattgagcctgtttctctgcgcgacgttcgcggcggcgtgtttgtgcatccatctggattctcctgtcagttagctttggtggtgtgtggcagttgtagtcctgaacgaaaaccccccgcgattggcacattggcagctaatccggaatcgcacttacggccaatgcttcgtttcgtatcacacaccccaaagccttctgctttgaatgctgcccttcttcagggcttaatttttaagagcgtcaccttcatggtggtcagtgcgtcctgctgatgtgctcagtatcaccgccagtggtatttatgtcaacaccgccagagataatttatcaccgcagatggttatctgtatgttttttatatgaatttattttttgcaggggggcattgtttggtaggtgagagatctgaattgctatgtttagtgagttgtatctatttatttttcaataaatacaattggttatgtgttttgggggcgatcgtgaggcaaagaaaacccggcgctgaggccgggttattcttgttctctggtcaaattatatagttggaaaacaaggatgcatatatgaatgaacgatgcagaggcaatgccgatggcgatagtgggtatcatgtagccgcttatgctggaaagaagcaataacccgcagaaaaacaaagctccaagctcaacaaaactaagggcatagacaataactaccgatgtcatatacccatactctctaatcttggccagtcggcgcgttctgcttccgattagaaacgtcaaggcagcaatcaggattgcaatcatggttcctgcatatgatgacaatgtcgccccaagaccatctctatgagctgaaaaagaaacaccaggaatgtagtggcggaaaaggagatagcaaatgcttacgataacgtaaggaattattactatgtaaacaccaggcatgattctgttccgcataattactcctgataattaatccttaactttgcccacctgccttttaaaacattccagtatatcacttttcattcttgcgtagcaatatgccatctcttcagctatctcagcattggtgaccttgttcagaggcgctgagagatggcctttttctgatagataatgttctgttaaaatatctccggcctcatcttttgcccgcaggctaatgtctgaaaattgaggtgacgggttaaaaataatatccttggcaaccttttttatatcccttttaaattttggcttaatgactatatccaatgagtcaaaaagctccccttcaatatctgttgcccctaagacctttaatatatcgccaaatacaggtagcttggcttctaccttcaccgttgttcggccgatgaaatgcatatgcataacatcgtctttggtggttcccctcatcagtggctctatctgaacgcgctctccactgcttaatgacattcctttcccgattaaaaaatctgtcagatcggatgtggtcggcccgaaaacagttctggcaaaaccaatggtgtcgccttcaacaaacaaaaaagatgggaatcccaatgattcgtcatctgcgaggctgttcttaatatcttcaactgaagctttagagcgatttatcttctgaaccagactcttgtcatttgttttggtaaagagaaaagtttttccatcgattttatgaatatacaaataattggagccaacctgcaggtgatgattatcagccagcagagaattaaggaaaacagacaggtttattgagcgcttatctttccctttatttttgctgcggtaagtcgcataaaaaccattcttcataattcaatccatttactatgttatgttctgaggggagtgaaaattcccctaattcgatgaagattcttgctcaattgttatcagctatgcgccgaccagaacaccttgccgatcagccaaacgtctcttcaggccactgactagcgataactttccccacaacggaacaactctcattgcatgggatcattgggtactgtgggtttagtggttgtaaaaacacctgaccgctatccctgatcagtttcttgaaggtaaactcatcacccccaagtctggctatgcagaaatcacctggctcaacagcctgctcagggtcaacgagaattaacattccgtcaggaaagcttggcttggagcctgttggtgcggtcatggaattaccttcaacctcaagccagaatgcagaatcactggcttttttggttgtgcttacccatctctccgcatcacctttggtaaaggttctaagcttaggtgagaacatccctgcctgaacatgagaaaaaacagggtactcatactcacttctaagtgacggctgcatactaaccgcttcatacatctcgtagatttctctggcgattgaagggctaaattcttcaacgctaactttgagaatttttgtaagcaatgcggcgttataagcatttaatgcattgatgccattaaataaagcaccaacgcctgactgccccatccccatcttgtctgcgacagattcctgggataagccaagttcatttttctttttttcataaattgctttaaggcgacgtgcgtcctcaagctgctcttgtgttaatggtttcttttttgtgctcatacgttaaatctatcaccgcaagggataaatatctaacaccgtgcgtgttgactattttacctctggcggtgataatggttgcatgtactaaggaggttgtatggaacaacgcataaccctgaaagattatgcaatgcgctttgggcaaaccaagacagctaaagatctcggcgtatatcaaagcgcgatcaacaaggccattcatgcaggccgaaagatttttttaactataaacgctgatggaagcgtttatgcggaagaggtaaagcccttcccgagtaacaaaaaaacaacagcataaataaccccgctcttacacattccagccctgaaaaagggcatcaaattaaaccacacctatggtgtatgcatttatttgcatacattcaatcaattgttatctaaggaaatacttacatatggttcgtgcaaacaaacgcaacgaggctctacgaatcgagagtgcgttgcttaacaaaatcgcaatgcttggaactgagaagacagcggaagctgtgggcgttgataagtcgcagatcagcaggtggaagagggactggattccaaagttctcaatgctgcttgctgttcttgaatggggggtcgttgacgacgacatggctcgattggcgcgacaagttgctgcgattctcaccaataaaaaacgcccggcggcaaccgagcgttctgaacaaatccagatggagttctgaggtcattactggatctatcaacaggagtcattatgacaaatacagcaaaaatactcaacttcggcagaggtaactttgccggacaggagcgtaatgtggcagatctcgatgatggttacgccagactatcaaatatgctgcttgaggcttattcgggcgcagatctgaccaagcgacagtttaaagtgctgcttgccattctgcgtaaaacctatgggtggaataaaccaatggacagaatcaccgattctcaacttagcgagattacaaagttacctgtcaaacggtgcaatgaagccaagttagaactcgtcagaatgaatattatcaagcagcaaggcggcatgtttggaccaaataaaaacatctcagaatggtgcatccctcaaaacgagggaaaatcccctaaaacgagggataaaacatccctcaaattgggggattgctatccctcaaaacagggggacacaaaagacactattacaaaagaaaaaagaaaagattattcgtcagagaattctggcgaatcctctgaccagccagaaaacgacctttctgtggtgaaaccggatgctgcaattcagagcggcagcaagtgggggacagcagaagacctgaccgccgcagagtggatgtttgacatggtgaagactatcgcaccatcagccagaaaaccgaattttgctgggtgggctaacgatatccgcctgatgcgtgaacgtgacggacgtaaccaccgcgacatgtgtgtgctgttccgctgggcatgccaggacaacttctggtccggtaacgtgctgagcccggccaaactccgcgataagtggacccaactcgaaatcaaccgtaacaagcaacaggcaggcgtgacagccagcaaaccaaaactcgacctgacaaacacagactggatttacggggtggatctatgaaaaacatcgccgcacagatggttaactttgaccgtgagcagatgcgtcggatcgccaacaacatgccggaacagtacgacgaaaagccgcaggtacagcaggtagcgcagatcatcaacggtgtgttcagccagttactggcaactttcccggcgagcctggctaaccgtgaccagaacgaagtgaacgaaatccgtcgccagtgggttctggcttttcgggaaaacgggatcaccacgatggaacaggttaacgcaggaatgcgcgtagcccgtcggcagaatcgaccatttctgccatcacccgggcagtttgttgcatggtgccgggaagaagcatccgttaccgccggactgccaaacgtcagcgagctggttgatatggtttacgagtattgccggaagcgaggcctgtatccggatgcggagtcttatccgtggaaatcaaacgcgcactactggctggttaccaacctgtatcagaacatgcgggccaatgcgcttactgatgcggaattacgccgtaaggccgcagatgagcttgtccatatgactgcgagaattaaccgtggtgaggcgatccctgaaccagtaaaacaacttcctgtcatgggcggtagacctctaaatcgtgcacaggctctggcgaagatcgcagaaatcaaagctaagttcggactgaaaggagcaagtgtatgacgggcaaagaggcaattattcattacctggggacgcataatagcttctgtgcgccggacgttgccgcgctaacaggcgcaacagtaaccagcataaatcaggccgcggctaaaatggcacgggcaggtcttctggttatcgaaggtaaggtctggcgaacggtgtattaccggtttgctaccagggaagaacgggaaggaaagatgagcacgaacctggtttttaaggagtgtcgccagagtgccgcgatgaaacgggtattggcggtatatggagttaaaagatgaccatctacattactgagctaataacaggcctgctggtaatcgcaggcctttttatttgggggagagggaagtcatgaaaaaactaacctttgaaattcgatctccagcacatcagcaaaacgctattcacgcagtacagcaaatccttccagacccaaccaaaccaatcgtagtaaccattcaggaacgcaaccgcagcttagaccaaaacaggaagctatgggcctgcttaggtgacgtctctcgtcaggttgaatggcatggtcgctggctggatgcagaaagctggaagtgtgtgtttaccgcagcattaaagcagcaggatgttgttcctaaccttgccgggaatggctttgtggtaataggccagtcaaccagcaggatgcgtgtaggcgaatttgcggagctattagagcttatacaggcattcggtacagagcgtggcgttaagtggtcagacgaagcgagactggctctggagtggaaagcgagatggggagacagggctgcatgataaatgtcgttagtttctccggtggcaggacgtcagcatatttgctctggctaatggagcaaaagcgacgggcaggtaaagacgtgcattacgttttcatggatacaggttgtgaacatccaatgacatatcggtttgtcagggaagttgtgaagttctgggatataccgctcaccgtattgcaggttgatatcaacccggagcttggacagccaaatggttatacggtatgggaaccaaaggatattcagacgcgaatgcctgttctgaagccatttatcgatatggtaaagaaatatggcactccatacgtcggcggcgcgttctgcactgacagattaaaactcgttcccttcaccaaatactgtgatgaccatttcgggcgagggaattacaccacgtggattggcatcagagctgatgaaccgaagcggctaaagccaaagcctggaatcagatatcttgctgaactgtcagactttgagaaggaagatatcctcgcatggtggaagcaacaaccattcgatttgcaaataccggaacatctcggtaactgcatattctgcattaaaaaatcaacgcaaaaaatcggacttgcctgcaaagatgaggagggattgcagcgtgtttttaatgaggtcatcacgggatcccatgtgcgtgacggacatcgggaaacgccaaaggagattatgtaccgaggaagaatgtcgctggacggtatcgcgaaaatgtattcagaaaatgattatcaagccctgtatcaggacatggtacgagctaaaagattcgataccggctcttgttctgagtcatgcgaaatatttggagggcagcttgatttcgacttcgggagggaagctgcatgatgcgatgttatcggtgcggtgaatgcaaagaagataaccgcttccgaccaaatcaaccttactggaatcgatggtgtctccggtgtgaaagaacaccaacaggggtgttaccactaccgcaggaaaaggaggacgtgtggcgagacagcgacgaagtatcaccgacataatctgcgaaaactgcaaataccttccaacgaaacgcaccagaaataaacccaagccaatcccaaaagaatctgacgtaaaaaccttcaactacacggctcacctgtgggatatccggtggctaagacgtcgtgcgaggaaaacaaggtgattgaccaaaatcgaagttacgaacaagaaagcgtcgagcgagctttaacgtgcgctaactgcggtcagaagctgcatgtgctggaagttcacgtgtgtgagcactgctgcgcagaactgatgagcgatccgaatagctcgatgcacgaggaagaagatgatggctaaaccagcgcgaagacgatgtaaaaacgatgaatgccgggaatggtttcaccctgcattcgctaatcagtggtggtgctctccagagtgtggaaccaagatagcactcgaacgacgaagtaaagaacgcgaaaaagcggaaaaagcagcagagaagaaacgacgacgagaggagcagaaacagaaagataaacttaagattcgaaaactcgccttaaagccccgcagttactggattaaacaagcccaacaagccagga

SEQ ID NO: 24 - DNA, 15 bp, Artificial Sequence
  Adaptor portion G of Fig 5
ttgaccgctcgcctc